European Patent Application EP 4 455 289 A1, published October 30, 2024. Title: AMYLASE-CONTAINING DETERGENT COMPOSITION. Applicant: KAO CORPORATION. The sequence listing filed with the application follows.

SEQUENCE LISTING (11 sequences)

SEQ ID NO: 1 - DNA, 1458 bp, synthetic construct
  source 1..1458: mol_type = other DNA
  CDS 1..1455
gcagctcaaaacggtacgatgatgcagtactttgaatggtatgtaccgaatgatggtcagcattggaatcgtctgcggaacgatgcagcctacttgaaatccatcggtgtgtcagctatctggacacctcctgcttacaaaggcacaagccagaacgatgttggctatggagcatatgacctgtacgatttaggagaattcaaccagaaaggcactattcgcaccaaatatggaacgaaagctgaactgaaaagcgcggtatcgactctcaagtctaatgggattcaagtgtatggagatgtcgtcatgaatcataaaggcggtgccgattacacagagaatgtaacagctgtggaagtcaatccgagcaatcgcaatcaagaaacatccgatgagtatacgatccaagcatggacaggattcaacttccctgggcgaggcacaacccatagtccgtttaagtggcagtggtatcattttgatggaactgactgggatcagtctcggaatgcgagcagaatcttcaaatttcgtgggacaggaaaagcatgggattgggaagtatcatcggagaatgggaattacgactatcttatgtacgccgatttagactttgatcatcctgatgttagaaatgagatgaagaattggggcgtgtggtacgcgaatgaagttggcttggacggatttaggctggatgcggttaagcacataaagcatagctatctgggcgattgggtgaaccatgtcagaactaagacgggaaaagagatgtttacagttgctgaatattggcaaaacgacgtcaatgccattaataactatttagccaaagtgaactataatcactctgtctttgatgcgcctttgcattacaactttcactatgcaagccagtcaggaggtaactacgacatgcgtaacttattgaacggcacagtcgtggctgctcatccgacaaaagcagttacccttgtcgaaaatcatgacagtcaaccgggacaatctctggagtcagtcgttcaaccgtggtttaagccccttgcctatgcgtttatcctcacacgagcagaaggttatccaagtatcttttatggggatatgtatgggactaagggaaactcatcgtacgaaattccagcactcaaaaccaaaattgaaccgttactgaaagcacgcaaggattatgcctatggtacgcagcacaactatatggaccactgggatgttataggttggaccagagaaggtgactccacgaaagaaaaatctggccttgcgacgcttgtgacagacggggcaggcgggtctaaatggatgtatgtaggcaaacagaatgctggcgaagtttggtatgacatcacaggcaatagaacggataaaatcaccattaatacagatggctggggaaacttccaagtaaacggaggctcagtctccgtgtacgttcaacagtaa

SEQ ID NO: 2 - protein, 485 aa, Bacillus sp. YR288
AAQNGTMMQYFEWYVPNDGQHWNRLRNDAAYLKSIGVSAIWTPPAYKGTSQNDVGYGAYDLYDLGEFNQKGTIRTKYGTKAELKSAVSTLKSNGIQVYGDVVMNHKGGADYTENVTAVEVNPSNRNQETSDEYTIQAWTGFNFPGRGTTHSPFKWQWYHFDGTDWDQSRNASRIFKFRGTGKAWDWEVSSENGNYDYLMYADLDFDHPDVRNEMKNWGVWYANEVGLDGFRLDAVKHIKHSYLGDWVNHVRTKTGKEMFTVAEYWQNDVNAINNYLAKVNYNHSVFDAPLHYNFHYASQSGGNYDMRNLLNGTVVAAHPTKAVTLVENHDSQPGQSLESVVQPWFKPLAYAFILTRAEGYPSIFYGDMYGTKGNSSYEIPALKTKIEPLLKARKDYAYGTQHNYMDHWDVIGWTREGDSTKEKSGLATLVTDGAGGSKWMYVGKQNAGEVWYDITGNRTDKITINTDGWGNFQVNGGSVSVYVQQ

SEQ ID NO: 3 - DNA, 1452 bp, synthetic construct
  source 1..1452: mol_type = other DNA
  CDS 1..1449
gcagctcaaaacggtacgatgatgcagtactttgaatggtatgtaccgaatgatggtcagcattggaatcgtctgcggaacgatgcagcctacttgaaatccatcggtgtgtcagctatctggacacctcctgcttacaaaggcacaagccagaacgatgttggctatggagcatatgacctgtacgatttaggagaattcaaccagaaaggcactattcgcaccaaatatggaacgaaagctgaactgaaaagcgcggtatcgactctcaagtctaatgggattcaagtgtatggagatgtcgtcatgaatcataaaggcggtgccgattacacagagaatgtaacagctgtggaagtcaatccgagcaatcgcaatcaagaaacatccgatgagtatacgatccaagcatggacaggattcaacttccctgggcgaggcacaacccatagtccgtttaagtggcagtggtatcattttgatggaactgactgggatcagtctcggaatgcgagcagaatcttcaaatttgggggaaaagcatgggattgggaagtatcatcggagaatgggaattacgactatcttatgtacgccgatttagactttgatcatcctgatgttagaaatgagatgaagaattggggcgtgtggtacgcgaatgaagttggcttggacggatttaggctggatgcggttaagcacataaagcatagctatctgggcgattgggtgaaccatgtcagaactaagacgggaaaagagatgtttacagttgctgaatattggcaaaacgacgtcaatgccattaataactatttagccaaagtgaactataatcactctgtctttgatgcgcctttgcattacaactttcactatgcaagccagtcaggaggtaactacgacatgcgtaacttattgaacggcacagtcgtggctgctcatccgacaaaagcagttacccttgtcgaaaatcatgacagtcaaccgggacaatctctggagtcagtcgttcaaccgtggtttaagccccttgcctatgcgtttatcctcacacgagcagaaggttatccaagtatcttttatggggatatgtatgggactaagggaaactcatcgtacgaaattccagcactcaaaaccaaaattgaaccgttactgaaagcacgcaaggattatgcctatggtacgcagcacaactatatggaccactgggatgttataggttggaccagagaaggtgactccacgaaagaaaaatctggccttgcgacgcttgtgacagacggggcaggcgggtctaaatggatgtatgtaggcaaacagaatgctggcgaagtttggtatgacatcacaggcaatagaacggataaaatcaccattaatacagatggctggggaaacttccaagtaaacggaggctcagtctccgtgtacgttcaacagtaa

SEQ ID NO: 4 - protein, 483 aa, synthetic construct
AAQNGTMMQYFEWYVPNDGQHWNRLRNDAAYLKSIGVSAIWTPPAYKGTSQNDVGYGAYDLYDLGEFNQKGTIRTKYGTKAELKSAVSTLKSNGIQVYGDVVMNHKGGADYTENVTAVEVNPSNRNQETSDEYTIQAWTGFNFPGRGTTHSPFKWQWYHFDGTDWDQSRNASRIFKFGGKAWDWEVSSENGNYDYLMYADLDFDHPDVRNEMKNWGVWYANEVGLDGFRLDAVKHIKHSYLGDWVNHVRTKTGKEMFTVAEYWQNDVNAINNYLAKVNYNHSVFDAPLHYNFHYASQSGGNYDMRNLLNGTVVAAHPTKAVTLVENHDSQPGQSLESVVQPWFKPLAYAFILTRAEGYPSIFYGDMYGTKGNSSYEIPALKTKIEPLLKARKDYAYGTQHNYMDHWDVIGWTREGDSTKEKSGLATLVTDGAGGSKWMYVGKQNAGEVWYDITGNRTDKITINTDGWGNFQVNGGSVSVYVQQ

SEQ ID NO: 5 - protein, 269 aa, Bacillus clausii
AQSVPWGISRVQAPAAHNRGLTGSGVKVAVLDTGISTHPDLNIRGGASFVPGEPSTQDGNGHGTHVAGTIAALNNSIGVLGVAPSAELYAVKVLGASGSGSVSSIAQGLEWAGNNGMHVANLSLGSPSPSATLEQAVNSATSRGVLVVAASGNSGAGSISYPARYANAMAVGATDQNNNRASFSQYGAGLDIVAPGVNVQSTYPGSTYASLNGTSMATPHVAGAAALVKQKNPSWSNVQIRNHLKNTATSLGSTNLYGSGLVNAEAATR

SEQ ID NO: 6 - protein, 275 aa, Bacillus amyloliquefaciens [sequence omitted]

SEQ ID NO: 7 - protein, 269 aa, Bacillus lentus
AQSVPWGISRVQAPAAHNRGLTGSGVKVAVLDTGISTHPDLNIRGGASFVPGEPSTQDGNGHGTHVAGTIAALNNSIGVLGVAPSAELYAVKVLGADGRGAISSIAQGLEWAGNNGMHVANLSLGSPSPSATLEQAVNSATSRGVLVVAASGNSGASSISYPARYANAMAVGATDQNNNRASFSQYGAGLDIVAPGVNVQSTYPGSTYASLNGTSMATPHVAGAAALVKQKNPSWSNVQIRNHLKNTATSLGSTNLYGSGLVNAEAATR

SEQ ID NO: 8 - protein, 434 aa, Bacillus sp.
NDVARGIVKADVAQSSYGLYGQGQIVAVADTGLDTGRNDSSMHEAFRGKITALYALGRTNNANDTNGHGTHVAGSVLGNGSTNKGMAPQANLVFQSIMDSGGGLGGLPSNLQTLFSQAYSAGARIHTNSWGAAVNGAYTTDSRNVDDYVRKNDMTILFAAGNEGPNGGTISAPGTAKNAITVGATENLRPSFGSYADNINHVAQFSSRGPTKDGRIKPDVMAPGTFILSARSSLAPDSSFWANHDSKYAYMGGTSMATPIVAGNVAQLREHFVKNRGITPKPSLLKAALIAGAADIGLGYPNGNQGWGRVTLDKSLNVAYVNESSSLSTSQKATYSFTATAGKPLKISLVWSDAPASTTASVTLVNDLDLVITAPNGTQYVGNDFTSPYNDNWDGRNNVENVFINAPQSGTYTIEVQAYNVPVGPQTFSLAIVN

SEQ ID NO: 9 - protein, 311 aa, Bacillus sp [sequence omitted]

SEQ ID NO: 10 - protein, 300 aa, Bacillus amyloliquefacience
AATTGTGTTLKGKTVSLNISSESGKYVLRDLSKPTGTQIITYDLQNREYNLPGTLVSSTTNQFTTSSQRAAVDAHYNLGKVYDYFYQKFNRNSYDNKGGKIVSSVHYGSRYNNAAWIGDQMIYGDGDGSFFSPLSGSMDVTAHEMTHGVTQETANLNYENQPGALNESFSDVFGYFNDTEDWDIGEDITVSQPALRSLSNPTKYGQPDNFKNYKNLPNTDAGDYGGVHTNSGIPNKAAYNTITKIGVNKAEQIYYRALTVYLTPSSTFKDAKAALIQSARDLYGSQDAASVEAAWNAVGL

SEQ ID NO: 11 - protein, 300 aa, Bacillus subtilis
AAATGSGTTLKGATVPLNISYEGGKYVLRDLSKPTGTQIITYDLQNRQSRLPGTLVSSTTKTFTSSSQRAAVDAHYNLGKVYDYFYSNFKRNSYDNKGSKIVSSVHYGTQYNNAAWTGDQMIYGDGDGSFFSPLSGSLDVTAHEMTHGVTQETANLIYENQPGALNESFSDVFGYFNDTEDWDIGEDITVSQPALRSLSNPTKYNQPDNYANYRNLPNTDEGDYGGVHTNSGIPNKAAYNTITKLGVSKSQQIYYRALTTYLTPSSTFKDAKAALIQSARDLYGSTDAAKVEAAWNAVGL